European Patent Specification EP 4 051 810 B1, published August 28, 2024. Title: METHOD FOR MAPPING ROLLING CIRCLE AMPLIFICATION PRODUCTS. Applicant: Pixelgen Technologies AB Fredriksson, Simon. The sequence listing filed with the application follows.

SEQUENCE LISTING (20 sequences)

SEQ ID NO: 1 - DNA, 27 bp, Artificial sequence
  synthetic sequence
tcgggatcggcatcgacgcctaaaaaa

SEQ ID NO: 2 - DNA, 80 bp, Artificial sequence
  synthetic sequence
  misc_feature (51)..(52): TP-BC is present between the nucleotides.
tgaaggtagacggaggatttataaaaaaataggcgtcgatgccgatcccgaaaaaaaacaacatcagtattcccaggcta

SEQ ID NO: 3 - DNA, 98 bp, Artificial sequence
  synthetic sequence
  misc_feature (39)..(60): n is a, c, g, or t
tggttcgcaggatgaggccgggagtctaactcaaatacnnnnnnnnnnnnnnnnnnnnnntgaaggtagacggaggatttatcgcttcggtgagatag

SEQ ID NO: 4 - DNA, 32 bp, Artificial sequence
  synthetic sequence
ctcatcctgcgaaccactatctcaccgaagcg

SEQ ID NO: 5 - DNA, 98 bp, Artificial sequence
  synthetic sequence
  misc_feature (39)..(60): n is a, c, g, or t
ctatctcaccgaagcgataaatcctccgtctaccttcannnnnnnnnnnnnnnnnnnnnngtatttgagttagactcccggcctcatcctgcgaacca

SEQ ID NO: 6 - DNA, 22 bp, Artificial sequence
  synthetic sequence
gccgggagtctaactcaaatac

SEQ ID NO: 7 - DNA, 98 bp, Artificial sequence
  synthetic sequence
  misc_feature (39)..(60): n is a, c, g, or t
tagtgagtgtacggaccaacatcagtattcccaggctannnnnnnnnnnnnnnnnnnnnngtgctgaccaatcgaccaagatcgcctagtctctacta

SEQ ID NO: 8 - DNA, 32 bp, Artificial sequence
  synthetic sequence
gtccgtacactcactatagtagagactaggcg

SEQ ID NO: 9 - DNA, 98 bp, Artificial sequence
  synthetic sequence
  misc_feature (39)..(60): n is a, c, g, or t
tagtagagactaggcgatcttggtcgattggtcagcacnnnnnnnnnnnnnnnnnnnnnntagcctgggaatactgatgttggtccgtacactcacta

SEQ ID NO: 10 - DNA, 22 bp, Artificial sequence
  synthetic sequence
gtgctgaccaatcgaccaagat

SEQ ID NO: 11 - DNA, 22 bp, Artificial sequence
  synthetic sequence
gtatttgagttagactcccggc

SEQ ID NO: 12 - DNA, 22 bp, Artificial sequence
  synthetic sequence
atcttggtcgattggtcagcac

SEQ ID NO: 13 - DNA, 124 bp, Artificial sequence
  synthetic sequence
  misc_feature (22)..(22): A randomly generated UMI barcode "Nx22" is present between the nucleotides
  misc_feature (102)..(103): A randomly generated UMI barcode "Nx22" is present between the nucleotides
gccgggagtctaactcaaatactgaaggtagacggaggatttataaaaaaataggcgtcgatgccgatcccgaaaaaaaacaacatcagtattcccaggctagtgctgaccaatcgaccaagat

SEQ ID NO: 14 - DNA, 27 bp, Artificial sequence
  synthetic sequence
catttcagacggtccggtgccaaaaaa

SEQ ID NO: 15 - DNA, 80 bp, Artificial sequence
  synthetic sequence
acataggagacaattgaatagcaaaaaaatggcaccggaccgtctgaaatgaaaaaaaatgaattacgcgcgctcagaca

SEQ ID NO: 16 - DNA, 51 bp, Artificial sequence
  synthetic sequence
ctagacgctgtagttctgtagcaaaaaaacaacatcagtattcccaggcta

SEQ ID NO: 17 - DNA, 44 bp, Artificial sequence
  synthetic sequence
gctattcaattgtctcctatgtcgtttcaatacgttgcatgatc

SEQ ID NO: 18 - DNA, 44 bp, Artificial sequence
  synthetic sequence
gctacagaactacagcgtctagtgtctgagcgcgcgtaattcat

SEQ ID NO: 19 - DNA, 228 bp, Artificial sequence
  synthetic sequence
  misc_feature (22)..(23): A randomly generated UMI barcode "Nx22" is present between the nucleotides
  misc_feature (205)..(206): A randomly generated UMI barcode "Nx22" is present between the nucleotides
gccgggagtctaactcaaatacntgaaggtagacggaggatttataaaaaaagatcatgcaacgtattgaaacgacataggagacaattgaatagcaaaaaaatggcaccggaccgtctgaaatgaaaaaaaatgaattacgcgcgctcagacactagacgctgtagttctgtagcaaaaaaacaacatcagtattcccaggctangtgctgaccaatcgaccaagat

SEQ ID NO: 20 - DNA, 51 bp, Artificial sequence
  synthetic sequence
tgaaggtagacggaggatttataaaaaaagatcatgcaacgtattgaaacg